European Patent Application EP 4 249 590 A1, published September 27, 2023. Title: Heat Resistant Protein-Glutaminase. Applicant: AMANO ENZYME INC. The sequence listing filed with the application follows.

SEQUENCE LISTING (6 sequences)

SEQ ID NO: 1 - protein, 319 aa, Chryseobacterium sp.
MKKFLLSMMVFVTMLSFNACSDSAANQDPNLVAKESNEIAMKDFGKTVPVGIEKEEGKFKVSFMVSAQPYHIKDSKENAGYISMIRQAVENETPVHIFLKTNTTEIAKVDKPTDDDIRYFKSVFNKEERGDSKKAVSVIPNLATLNSLFTQIKNQACGTSTASSPCITFRYPVDGCYARAHKMRQILLNAGYDCEKQFVYGNLRASTGTCCVSWVYHVAILVSFKNASGIVEKRIIDPSLFSSGPVTDAAWRAACTNTSCGSASVSSYANTAGNVYYRSPSGSLLYDNNYVNTNCVLNIFSSLSGCSPSPAPSVASCGF

SEQ ID NO: 2 - protein, 319 aa, Chryseobacterium sp.
MKKFLLSMMVFVTVLSFNSCSDSSANQDPNLVAKESNEIAMKDFGKTVPVGIEKEDGKFKVSFIVSAQPYQIKDTKENAGYISMIKEAVENETPVQVFLKANSNEIAKVDKATADDIRYFKSVFNKEERGDSRKAVSVIPNLATLNSLFTQIKNQACGTSTASSPCITFRYPVDGCYARAHKMRQILLNAGYDCEKQFVYGNLRASTGTCCVSWVYHVAILVSFKNASGIVEKRIIDPSLFSSGPVTDTAWRAACTNTSCGSASVSSYANTAGNVYYRSPSGSLLYDNNYVNTNCVLNIFSSLSGCSPSPAPSVASCGF

SEQ ID NO: 3 - DNA, 960 bp, Chryseobacterium sp.
atgaaaaaatttctgttatccatgatggtattcgtgacgatgctgtcattcaatgcctgttcagattcagctgccaatcaggatcccaatcttgttgctaaagagtctaatgaaatcgccatgaaagatttcggtaaaactgttccggtagggattgaaaaagaagagggaaaatttaaagtctcttttatggtgagtgctcagccataccacattaaagacagtaaggaaaatgcaggttatatttctatgatcagacaagccgttgaaaacgaaactcctgttcatattttcctgaaaaccaacaccactgaaattgcaaaagtagataaacctactgatgatgatatccgttatttcaaatctgttttcaataaagaagagagaggagacagcaaaaaagcagtgagtgttattcctaacctggcaacactgaacagcttatttacgcagattaaaaaccaggcttgcggtacttctacagcatcttctccatgtatcactttcagatatccggtggatggatgttatgcaagagctcacaaaatgagacagatcctccttaatgcaggctacgactgtgaaaagcagttcgtttacggaaacctgagagcttctacaggaacttgctgcgtatcatgggtatatcacgtagccatattggtaagcttcaaaaatgcttccggaattgttgagaaaagaatcatcgatccttcactattctccagcggacccgtaactgacgcagcatggagagccgcttgtaccaacacaagctgtggatctgcttctgtatcttcttatgccaatacagcaggaaacgtgtactacagaagtccatcaggatctttactgtatgataacaattatgtaaataccaattgtgtattgaatatattctcatccctttcaggatgttctccttctcctgcaccaagtgtagcgagctgcggattttaa

SEQ ID NO: 4 - DNA, 960 bp, Chryseobacterium sp.
atgaaaaaatttcttttatccatgatggtattcgtgacggtactttcatttaactcctgttcggattcaagtgccaatcaggatccgaatcttgttgctaaagagtctaatgaaattgctatgaaagactttggtaaaactgttccggtagggatagaaaaagaggatggaaagtttaaagtttcctttatagtttcagcgcagccgtatcaaattaaagatacaaaagaaaatgcgggatatatctccatgatcaaagaggctgtagaaaatgaaactcctgttcaggttttcctgaaagccaattctaacgaaatcgcaaaggtagacaaagcaacagcggatgacatccgttatttcaaatctgttttcaacaaagaagagagaggcgacagcagaaaagctgtgagcgttattcctaatcttgcaacgctgaacagcttattcactcagatcaaaaaccaggcttgcggaacttctacagcatcttcaccgtgtatcacattcagatatcctgtggatggatgctatgcgagagctcacaaaatgagacaaatccttttgaatgcaggctacgactgtgaaaaacagttcgtttacgggaacctaagagcatctacaggaacatgctgtgtgtcttgggtatatcacgtagccattttggtaagcttcaaaaatgcttccggaattgttgagaaaagaattattgatccgtcactattctccagcggacctgtaacagatactgcatggagagccgcatgtaccaacacaagctgtggatctgcttctgtttcttcttatgccaatacagcaggaaatgtatactacagaagcccatccggttctttattatatgataacaattatgtaaataccaactgtgtattgaacatattctcatccctttcaggatgttctccttcccctgcacctagtgtagcaagctgtggattttaa

SEQ ID NO: 5 - DNA, 1028 bp, Chryseobacterium sp.
caaaatagtgaactattatagttaaaaagttcactgaaaattaaccaccaaaatataaaaactatgaaaaaatttctgttatccatgatggtattcgtgacgatgctgtcattcaatgcctgttcagattcagctgccaatcaggatcccaatcttgttgctaaagagtctaatgaaatcgccatgaaagatttcggtaaaactgttccggtagggattgaaaaagaagagggaaaatttaaagtctcttttatggtgagtgctcagccataccacattaaagacagtaaggaaaatgcaggttatatttctatgatcagacaagccgttgaaaacgaaactcctgttcatattttcctgaaaaccaacaccactgaaattgcaaaagtagataaacctactgatgatgatatccgttatttcaaatctgttttcaataaagaagagagaggagacagcaaaaaagcagtgagtgttattcctaacctggcaacactgaacagcttatttacgcagattaaaaaccaggcttgcggtacttctacagcatcttctccatgtatcactttcagatatccggtggatggatgttatgcaagagctcacaaaatgagacagatcctccttaatgcaggctacgactgtgaaaagcagttcgtttacggaaacctgagagcttctacaggaacttgctgcgtatcatgggtatatcacgtagccatattggtaagcttcaaaaatgcttccggaattgttgagaaaagaatcatcgatccttcactattctccagcggacccgtaactgacgcagcatggagagccgcttgtaccaacacaagctgtggatctgcttctgtatcttcttatgccaatacagcaggaaacgtgtactacagaagtccatcaggatctttactgtatgataacaattatgtaaataccaattgtgtattgaatatattctcatccctttcaggatgttctccttctcctgcaccaagtgtagcgagctgcggattttaactaat

SEQ ID NO: 6 - DNA, 1029 bp, Chryseobacterium sp.
tagtgaactataaaaactaaaagttcactaaaaattaaccaccaaaatataaaaactatgaaaaaatttcttttatccatgatggtattcgtgacggtactttcatttaactcctgttcggattcaagtgccaatcaggatccgaatcttgttgctaaagagtctaatgaaattgctatgaaagactttggtaaaactgttccggtagggatagaaaaagaggatggaaagtttaaagtttcctttatagtttcagcgcagccgtatcaaattaaagatacaaaagaaaatgcgggatatatctccatgatcaaagaggctgtagaaaatgaaactcctgttcaggttttcctgaaagccaattctaacgaaatcgcaaaggtagacaaagcaacagcggatgacatccgttatttcaaatctgttttcaacaaagaagagagaggcgacagcagaaaagctgtgagcgttattcctaatcttgcaacgctgaacagcttattcactcagatcaaaaaccaggcttgcggaacttctacagcatcttcaccgtgtatcacattcagatatcctgtggatggatgctatgcgagagctcacaaaatgagacaaatccttttgaatgcaggctacgactgtgaaaaacagttcgtttacgggaacctaagagcatctacaggaacatgctgtgtgtcttgggtatatcacgtagccattttggtaagcttcaaaaatgcttccggaattgttgagaaaagaattattgatccgtcactattctccagcggacctgtaacagatactgcatggagagccgcatgtaccaacacaagctgtggatctgcttctgtttcttcttatgccaatacagcaggaaatgtatactacagaagcccatccggttctttattatatgataacaattatgtaaataccaactgtgtattgaacatattctcatccctttcaggatgttctccttcccctgcacctagtgtagcaagctgtggattttaattaatttataga